European Patent Application EP 4 317 431 A2, published February 7, 2024. Title: PREVENTING AND/OR TREATING AGENT FOR INFECTIOUS DISEASE OR INFLAMMATORY DISEASE. Applicant: A-CLIP INSTITUTE, CO., LTD. Application EP. The sequence listing filed with the application follows.

SEQUENCE LISTING (9 sequences)

SEQ ID NO: 1 - DNA, 303 bp, Homo sapiens
  misc_feature 1..303: note = Coding DNA sequence for human APOA2
  source 1..303: mol_type = genomic DNA
atgaagctgctcgcagcaactgtgctactcctcaccatctgcagccttgaaggagctttggttcggagacaggcaaaggagccatgtgtggagagcctggtttctcagtacttccagaccgtgactgactatggcaaggacctgatggagaaggtcaagagcccagagcttcaggccgaggccaagtcttactttgaaaagtcaaaggagcagctgacacccctgatcaagaaggctggaacggaactggttaacttcttgagctatttcgtggaacttggaacacagcctgccacccagtga

SEQ ID NO: 2 - protein, 100 aa, Homo sapiens
  REGION 1..100: note = MISC_FEATURE - Amino acid sequence of human APOA2
MKLLAATVLLLTICSLEGALVRRQAKEPCVESLVSQYFQTVTDYGKDLMEKVKSPELQAEAKSYFEKSKEQLTPLIKKAGTELVNFLSYFVELGTQPATQ

SEQ ID NO: 3 - DNA, 798 bp, synthetic construct
  misc_feature 1..798: note = DNA sequence coding VasAP antibody
  source 1..798: mol_type = other DNA
atggatttcggccttagctggattttcctggtagcgctgctgcgtggcgtacagtgccaagtacacttagtggagtctggtggtggcttggttcaaccgggtcgttctctgcggctctcatgtgcggtgagcggcttcacctttgcgtcctatgccatgcattgggtccgtcaggctcctggcaaagggctggaatgggtcgcagggatcagtaaggatgggagcaacaaacgtcatgccgatagcctcgaaggccgctttaccattagtcgcgataactcgaagaacaccctgtatctccaggttagtggcttacgcgcagaagataccgccgtttactattgtgcgcgctcacaagatccgacggacttcgattggcttctgtccgaacattggggtcagggtactctggtgacagtctcgtcagcgagcacaaaaggcccgtcggtgtttccgttagccccttgttctcgcagtacttccgagagtactgctgcactgggttgcctggtgaaagactacttcccggaaccggttaccgtgtcgtggaattcaggtgcactgacctctggagtccatacgtttcctgcggttttgcagtcgagcggcttgtactctctgagcagcgttgtgacggtgccgagctccaactttggaacccagacctatacgtgcaatgtggatcacaaaccctccaatacgaaggtagacaaaaccgtggctccaccagttgccggtccaagcgtctttctgtttccgcccaaaccgaaagacacacatcaccaccatcaccattaa

SEQ ID NO: 4 - protein, 265 aa, synthetic construct
  REGION 1..265: note = Amino acid sequence of VasAP antibody
MDFGLSWIFLVALLRGVQCQVHLVESGGGLVQPGRSLRLSCAVSGFTFASYAMHWVRQAPGKGLEWVAGISKDGSNKRHADSLEGRFTISRDNSKNTLYLQVSGLRAEDTAVYYCARSQDPTDFDWLLSEHWGQGTLVTVSSASTKGPSVFPLAPCSRSTSESTAALGCLVKDYFPEPVTVSWNSGALTSGVHTFPAVLQSSGLYSLSSVVTVPSSNFGTQTYTCNVDHKPSNTKVDKTVAPPVAGPSVFLFPPKPKDTHHHHHH

SEQ ID NO: 5 - DNA, 40 bp, synthetic construct
  misc_feature 1..40: note = Base sequence for PCR primer (pET32_Rq01OptEc_infF(Tm))
  source 1..40: mol_type = other DNA
tttaagaaggagatatacatatggatttcggcctcagctg

SEQ ID NO: 6 - DNA, 21 bp, synthetic construct
  misc_feature 1..21: note = Base sequence for PCR primer (Rq01_OptEc_cds_6HisStpcmpR)
  source 1..21: mol_type = other DNA
ttaatggtgatggtggtgatg

SEQ ID NO: 7 - DNA, 41 bp, synthetic construct
  misc_feature 1..41: note = Base sequence for PCR primer (His6StpCmp_pET32_110-129F)
  source 1..41: mol_type = other DNA
catcaccaccatcaccattaactgctaacaaagcccgaaag

SEQ ID NO: 8 - DNA, 20 bp, synthetic construct
  misc_feature 1..20: note = Base sequence for PCR primer (pET32vbRev693-712)
  source 1..20: mol_type = other DNA
atgtatatctccttcttaaa

SEQ ID NO: 9 - DNA, 20 bp, synthetic construct
  misc_feature 1..20: note = Base sequence for PCR primer (Rq01_OptEc_cds_F)
  source 1..20: mol_type = other DNA
atggatttcggcctcagctg